European Patent Application EP 4 218 771 A1, published August 2, 2023. Title: METHODS OF TREATING MOTOR NEURON DISEASES. Applicant: Yeda Research and Development Co. Ltd. The sequence listing filed with the application follows.

SEQUENCE LISTING (37 sequences)

SEQ ID NO: 1 - RNA, 110 nt, synthetic construct
  misc_feature 1..110: note = hsa-mir-218-1 complete seq
  source 1..110: mol_type = other RNA
gtgataatgtagcgagattttctgttgtgcttgatctaaccatgtggttgcgaggtatgagtaaaacatggttccgtcaagcaccatggaacgtcacgcagctttctaca

SEQ ID NO: 2 - RNA, 110 nt, synthetic construct
  misc_feature 1..110: note = hsa-mir-218-2 complete seq
  source 1..110: mol_type = other RNA
gaccagtcgctgcggggctttcctttgtgcttgatctaaccatgtggtggaacgatggaaacggaacatggttctgtcaagcaccgcggaaagcaccgtgctctcctgca

SEQ ID NO: 3 - RNA, 21 nt, synthetic construct
  misc_feature 1..21: note = hsa-miR-218
  source 1..21: mol_type = other RNA
ttgtgcttgatctaaccatgt

SEQ ID NO: 4 - RNA, 22 nt, synthetic construct
  misc_feature 1..22: note = hsa-miR-218-1*
  source 1..22: mol_type = other RNA
atggttccgtcaagcaccatgg

SEQ ID NO: 5 - RNA, 22 nt, synthetic construct
  misc_feature 1..22: note = hsa-miR-218-2*
  source 1..22: mol_type = other RNA
catggttctgtcaagcaccgcg

SEQ ID NO: 6 - DNA, 28 bp, synthetic construct
  misc_feature 1..28: note = Single strand DNA oligonucleotide
  source 1..28: mol_type = other DNA
cgtacgtaaagatggctgtgagggacag

SEQ ID NO: 7 - DNA, 33 bp, synthetic construct
  misc_feature 1..33: note = Single strand DNA oligonucleotide
  source 1..33: mol_type = other DNA
cgtacgtaagagagacccagtagaagcaaaaag

SEQ ID NO: 8-9 - skipped (2 entries)

SEQ ID NO: 10 - DNA, 21 bp, synthetic construct
  misc_feature 1..21: note = Single strand DNA oligonucleotide
  source 1..21: mol_type = other DNA
ttgtgcttgatctaaccatgt

SEQ ID NO: 11 - DNA, 21 bp, synthetic construct
  misc_feature 1..21: note = Single strand DNA oligonucleotide
  source 1..21: mol_type = other DNA
gatgacacgcaaattcgtgaa

SEQ ID NO: 12 - DNA, 22 bp, synthetic construct
  misc_feature 1..22: note = Single strand DNA oligonucleotide
  source 1..22: mol_type = other DNA
cgagatgctatgaaggagatgg

SEQ ID NO: 13 - DNA, 22 bp, synthetic construct
  misc_feature 1..22: note = Single strand DNA oligonucleotide
  source 1..22: mol_type = other DNA
gtaatccagcaggtcagcaaag

SEQ ID NO: 14 - DNA, 18 bp, synthetic construct
  misc_feature 1..18: note = Single strand DNA oligonucleotide
  source 1..18: mol_type = other DNA
cctttagtgggccctcgg

SEQ ID NO: 15 - DNA, 20 bp, synthetic construct
  misc_feature 1..20: note = Single strand DNA oligonucleotide
  source 1..20: mol_type = other DNA
gcctggagaaacctgccaag

SEQ ID NO: 16 - DNA, 20 bp, synthetic construct
  misc_feature 1..20: note = Single strand DNA oligonucleotide
  source 1..20: mol_type = other DNA
tgagcaggaggggaatcaga

SEQ ID NO: 17 - DNA, 20 bp, synthetic construct
  misc_feature 1..20: note = Single strand DNA oligonucleotide
  source 1..20: mol_type = other DNA
acacccttaccaagcggatg

SEQ ID NO: 18 - DNA, 19 bp, synthetic construct
  misc_feature 1..19: note = Single strand DNA oligonucleotide
  source 1..19: mol_type = other DNA
caagttcaccagcatccct

SEQ ID NO: 19 - DNA, 21 bp, synthetic construct
  misc_feature 1..21: note = Single strand DNA oligonucleotide
  source 1..21: mol_type = other DNA
cccgaaaatcttccctgctat

SEQ ID NO: 20 - DNA, 23 bp, synthetic construct
  misc_feature 1..23: note = Single strand DNA oligonucleotide
  source 1..23: mol_type = other DNA
acctgattctcacctacaatctg

SEQ ID NO: 21 - DNA, 21 bp, synthetic construct
  misc_feature 1..21: note = Single strand DNA oligonucleotide
  source 1..21: mol_type = other DNA
tcttccgtttcatcctctcct

SEQ ID NO: 22 - DNA, 19 bp, synthetic construct
  misc_feature 1..19: note = Single strand DNA oligonucleotide
  source 1..19: mol_type = other DNA
caccgtatcccacagcaat

SEQ ID NO: 23 - DNA, 21 bp, synthetic construct
  misc_feature 1..21: note = Single strand DNA oligonucleotide
  source 1..21: mol_type = other DNA
gaggtcattaggcttcgtctt

SEQ ID NO: 24 - DNA, 21 bp, synthetic construct
  misc_feature 1..21: note = Single strand DNA oligonucleotide
  source 1..21: mol_type = other DNA
cccagggtggcatttatgtct

SEQ ID NO: 25 - DNA, 20 bp, synthetic construct
  misc_feature 1..20: note = Single strand DNA oligonucleotide
  source 1..20: mol_type = other DNA
gggtgtgaaaaaggaccagc

SEQ ID NO: 26 - DNA, 20 bp, synthetic construct
  misc_feature 1..20: note = Single strand DNA oligonucleotide
  source 1..20: mol_type = other DNA
gtgggcatgagtggaacaca

SEQ ID NO: 27 - DNA, 20 bp, synthetic construct
  misc_feature 1..20: note = Single strand DNA oligonucleotide
  source 1..20: mol_type = other DNA
gatatagccaagacccggcg

SEQ ID NO: 28 - DNA, 20 bp, synthetic construct
  misc_feature 1..20: note = Single strand DNA oligonucleotide
  source 1..20: mol_type = other DNA
aagatgcgcctggatgtcaa

SEQ ID NO: 29 - DNA, 20 bp, synthetic construct
  misc_feature 1..20: note = Single strand DNA oligonucleotide
  source 1..20: mol_type = other DNA
atgctggaggcatcataggc

SEQ ID NO: 30 - DNA, 22 bp, synthetic construct
  misc_feature 1..22: note = Single strand DNA oligonucleotide
  source 1..22: mol_type = other DNA
gtcttccttttctctccttccc

SEQ ID NO: 31 - DNA, 27 bp, synthetic construct
  misc_feature 1..27: note = Single strand DNA oligonucleotide
  source 1..27: mol_type = other DNA
tcatcttcatcatctgctttatcaatg

SEQ ID NO: 32 - DNA, 20 bp, synthetic construct
  misc_feature 1..20: note = Single strand DNA oligonucleotide
  source 1..20: mol_type = other DNA
ctgacaccccatatcgacaa

SEQ ID NO: 33 - DNA, 22 bp, synthetic construct
  misc_feature 1..22: note = Single strand DNA oligonucleotide
  source 1..22: mol_type = other DNA
tccaaaaattgcgtagactcct

SEQ ID NO: 34 - DNA, 23 bp, synthetic construct
  misc_feature 1..23: note = Single strand DNA oligonucleotide
  source 1..23: mol_type = other DNA
catcaacagaaacaggactttgc

SEQ ID NO: 35 - DNA, 21 bp, synthetic construct
  misc_feature 1..21: note = Single strand DNA oligonucleotide
  source 1..21: mol_type = other DNA
gtgaaggaccgaagatagcag

SEQ ID NO: 36 - DNA, 21 bp, synthetic construct
  misc_feature 1..21: note = Single strand DNA oligonucleotide
  source 1..21: mol_type = other DNA
ggatgagacctgtactgtcat

SEQ ID NO: 37 - DNA, 21 bp, synthetic construct
  misc_feature 1..21: note = Single strand DNA oligonucleotide
  source 1..21: mol_type = other DNA
accttctacgtgaacctctac